European Patent Specification EP 3 171 891 B1, published September 10, 2025. Title: METHOD. Applicant: HANSA MEDICAL AB. The sequence listing filed with the application follows.

SEQUENCE LISTING (3 sequences)

SEQ ID NO: 1 - protein, 310 aa, Streptococcus pyogenes
DSFSANQEIRYSEVTPYHVTSVWTKGVTPPANFTQGEDVFHAPYVANQGWYDITKTFNGKDDLLCGAATAGNMLHWWFDQNKDQIKRYLEEHPEKQKINFNGEQMFDVKEAIDTKNHQLDSKLFEYFKEKAFPYLSTKHLGVFPDHVIDMFINGYRLSLTNHGPTPVKEGSKDPRGGIFDAVFTRGDQSKLLTSRHDFKEKNLKEISDLIKKELTEGKALGLSHTYANVRINHVINLWGADFDSNGNLKAIYVTDSDSNASIGMKKYFVGVNSAGKVAISAKEIKEDNIGAQVLGLFTLSTGQDSWNQTN

SEQ ID NO: 2 - protein, 959 aa, Streptococcus pyogenes
EEKTVQVQKGLPSIDSLHYLSENSKKEFKEELSKAGQESQKVKEILAKAQQADKQAQELAKMKIPEKIPMKPLHGPLYGGYFRTWHDKTSDPTEKDKVNSMGELPKEVDLAFIFHDWTKDYSLFWKELATKHVPKLNKQGTRVIRTIPWRFLAGGDNSGIAEDTSKYPNTPEGNKALAKAIVDEYVYKYNLDGLDVDVEHDSIPKVDKKEDTAGVERSIQVFEEIGKLIGPKGVDKSRLFIMDSTYMADKNPLIERGAPYINLLLVQVYGSQGEKGGWEPVSNRPEKTMEERWQGYSKYIRPEQYMIGFSFYEENAQEGNLWYDINSRKDEDKANGINTDITGTRAERYARWQPKTGGVKGGIFSYAIDRDGVAHQPKKYAKQKEFKDATDNIFHSDYSVSKALKTVMLKDKSYDLIDEKDFPDKALREAVMAQVGTRKGDLERFNGTLRLDNPAIQSLEGLNKFKKLAQLDLIGLSRITKLDRSVLPANMKPGKDTLETVLETYKKDNKEEPATIPPVSLKVSGLTGLKELDLSGFDRETLAGLDAATLTSLEKVDISGNKLDLAPGTENRQIFDTMLSTISNHVGSNEQTVKFDKQKPTGHYPDTYGKTSLRLPVANEKVDLQSQLLFGTVTNQGTLINSEADYKAYQNHKIAGRSFVDSNYHYNNFKVSYENYTVKVTDSTLGTTTDKTLATDKEETYKVDFFSPADKTKAVHTAKVIVGDEKTMMVNLAEGATVIGGSADPVNARKVFDGQLGSETDNISLGWDSKQSIIFKLKEDGLIKHWRFFNDSARNPETTNKPIQEASLQIFNIKDYNLDNLLENPNKFDDEKYWITVDTYSAQGERATAFSNTLNNITSKYWRVVFDTKGDRYSSPVVPELQILGYPLPNADTIMKTVTTAKELSQQKDKFSQKMLDELKIKEMALETSLNSKIFDVTAINANAGVLKDCIEKRQLLKK

SEQ ID NO: 3 - protein, 312 aa, Streptococcus pyogenes
DSFSANQEIRYSEVTPYHVTSVWTKGVTPPAKFTQGEDVFHAPYVANQGWYDITKTFNGKDDLLCGAATAGNMLHWWFDQNNEKIEAYLKKHPDKQKIMFGDQELLDVRKVINTKGDQTNSELFNYFRDKAFPGLSARRIGVMPDLVLDMFINGYYLNVYKTQTTDVNRTYQEKDRRGGIFDAVFTRGDQSKLLTSRHDFKEKTLKEISDLIKKELTEGKALGLSHTYANVRINHVINLWGADFDSNGNLEAIYVTDSDSNASIGMKKYFVGVNSAGKVAISAKEIKEDNIGAQVLGLFTLSTGQDSWNQTN